European Patent Application EP 4 477 740 A1, published December 18, 2024. Title: Production method of oligosaccharides containing Lewis X skeleton. Applicant: キリンホールディングス株式会社. The sequence listing filed with the application follows.

SEQUENCE LISTING (97 sequences)

SEQ ID NO: 1 - DNA, 969 bp, Parabacteroides goldsteinii JCM 13446
  source 1..969: mol_type = genomic DNA
atgaaaaagaaaatatactgcaactttgttgatttttggcttggttttaattataaaacttatttctggtatttgtcggatgaatacgatttgcagatagataaagagcatccggattatttattctattcctgttttggaaatgaacatttgttttatgaagactgtatccggattttttggagtgacgaaaacattatgcccgatcttaatatatgtgattatgccttaagtttgagtaatcttcaatgtgatgacagaacttttcggaaatatagtggatttctgtacagaaaggattttcacttggttttaccgcttttaaaagaagaagcgttgcttaaccgtaaattctgcaattttgtttattccaataatatttgtgccgtcccttatcgggagttgttctttaaaactttatccggttataaacggattgattccggtggtgcttttttgaataatatgggtaaaaaggtaggtgataagcaacagttcctacacgaatataaattcactttagcgattgaaaactcaagcatgccggggtatgtgactgaaaaaatcctggcaccgttcatggcacagtcgttaccgctatattggggcagccccactgtcagttcggattataatccgaactcgtttgttaatctgatgaattattcttccatggaagaagctgttgaggaggttatccgcctggacaaagacgatgccgcttatctggataaaatgatgacacccttttggccttatggcactaattttcaagaatttcgtgatagtgagataaaaaaaataaaagattttttcagtcatatttttgagcaaccattggataaagccggtcgtcgggtatgttatggccgtaataaaattactattcagaaacaaaggagatattatgctccgacatttcttgaattgtcaaaatctatgaccaaaaaactattgaaaaagaaataa

SEQ ID NO: 2 - protein, 322 aa, Parabacteroides goldsteinii JCM 13446
MKKKIYCNFVDFWLGFNYKTYFWYLSDEYDLQIDKEHPDYLFYSCFGNEHLFYEDCIRIFWSDENIMPDLNICDYALSLSNLQCDDRTFRKYSGFLYRKDFHLVLPLLKEEALLNRKFCNFVYSNNICAVPYRELFFKTLSGYKRIDSGGAFLNNMGKKVGDKQQFLHEYKFTLAIENSSMPGYVTEKILAPFMAQSLPLYWGSPTVSSDYNPNSFVNLMNYSSMEEAVEEVIRLDKDDAAYLDKMMTPFWPYGTNFQEFRDSEIKKIKDFFSHIFEQPLDKAGRRVCYGRNKITIQKQRRYYAPTFLELSKSMTKKLLKKK

SEQ ID NO: 3 - DNA, 1278 bp, Helicobacter pylori 26695
  source 1..1278: mol_type = genomic DNA
atgttccaacccctattagacgcctttatagaaagcgcttccattgaaaaaatggcctctaaatctccccccccccccctaaaaatcgctgtggcgaattggtggggagatgaagaaattaaagaatttaaaaagagcgttctttattttatcctaagccaacgctacgcaatcaccctccaccaaaaccccaatgaattttcagatctagtttttagcaatcctcttggagcggctagaaagattttatcttatcaaaacactaaacgagtgttttacaccggtgaaaacgaatcacctaatttcaacctctttgattacgccataggctttgatgaattggattttaatgatcgttatttgagaatgcctttgtattatgcccatttgcactataaagccgagcttgttaatgacaccactgcgccctacaaactcaaagacaacagcctttatgctttaaaaaaaccctctcatcattttaaagaaaaccaccctaatttgtgcgcagtagtgaatgatgagagcgatcttttaaaaagagggtttgccagttttgtagcgagcaacgctaacgctcctatgaggaacgctttttatgacgctctaaattccatagagccagttactgggggaggaagtgtgagaaacactttaggctataaggttggaaacaaaagcgagtttttaagccaatacaagttcaatctctgttttgaaaactcgcaaggttatggctatgtaaccgaaaaaatccttgatgcgtattttagccataccattcctatttattgggggagtcccagcgtggcgaaagattttaaccctaaaagttttgtgaatgtgcatgatttcaacaactttgatgaagcgattgattatatcaaatacctgcacacgcacccaaacgcttatttagacatgctctatgaaaaccctttaaacacccttgatgggaaagcttacttttaccaagatttgagttttaaaaaaatcctagatttttttaaaacgattttagaaaacgatacgatttatcacaaattctcaacatctttcatgtgggagtacgatctgcataagccgttagtatccattgatgatttgagggttaattatgatgatttgagggttaattatgaccggcttttacaaaacgcttcgcctttattagaactctctcaaaacaccacttttaaaatctatcgcaaagcttatcaaaaatccttgcctttgttgcgcgcggtgagaaagttggttaaaaaattgggtttgtaa

SEQ ID NO: 4 - protein, 425 aa, Helicobacter pylori 26695
MFQPLLDAFIESASIEKMASKSPPPPLKIAVANWWGDEEIKEFKKSVLYFILSQRYAITLHQNPNEFSDLVFSNPLGAARKILSYQNTKRVFYTGENESPNFNLFDYAIGFDELDFNDRYLRMPLYYAHLHYKAELVNDTTAPYKLKDNSLYALKKPSHHFKENHPNLCAVVNDESDLLKRGFASFVASNANAPMRNAFYDALNSIEPVTGGGSVRNTLGYKVGNKSEFLSQYKFNLCFENSQGYGYVTEKILDAYFSHTIPIYWGSPSVAKDFNPKSFVNVHDFNNFDEAIDYIKYLHTHPNAYLDMLYENPLNTLDGKAYFYQDLSFKKILDFFKTILENDTIYHKFSTSFMWEYDLHKPLVSIDDLRVNYDDLRVNYDRLLQNASPLLELSQNTTFKIYRKAYQKSLPLLRAVRKLVKKLGL

SEQ ID NO: 5 - DNA, 948 bp, Bacteroides nordii JCM 12987
  source 1..948: mol_type = genomic DNA
atgaaaactataaaagtaaaattcgttgatttctgggaaaactttgatccccaacacaacttcatagcaaatataatttctaagaaatatcggattgagcttagtgatactcctgattatctgttcttttcagtctttggatatgaaaatatagattatcacaattgtactaaaatattctactccggtgaaaacatcacgccagattttaatatctgcgactatgccattggctttaacttcctatcattcggtgacagatatatacgtatacctttttacacagcatatggtgtacagcaattagcagctcccaaagtgatagttcccgaagtggttcttaaccgtaaattctgtagtttcgtagtttctaatgccaaaggagctcccgaaagagaacgttttttccaactattgtcagaatacaaacaagtggattcgggaggccgctataaaaataatgtaggaggtccggttcccgataaaactgcttttatcaaggattacaaattcaatattgcatttgaaaatagcatgtgtgacggttataccactgaaaaaatcatggagccgatgcttgttaactccgtacctatctactggggtaataaacttattgaccgagatttcaacccggcttctttcatcaatgtctccagctattcttctttggaagaagcagtagagcacattgtccgactggatcagaatgatgatgagtacctttctctattatctgctccctggtttaatgaagagaattatctaaactgggaagaacaactgataaccttcttcgataatatcttcgaaaaacctctatccgaaagcagatatattccaactcacgggtatatccaaacttatcaatacagattgcaccgcatgatgagagataaattatttcgtaaacggatcaatccactgaaatggttttcttcgaagtga

SEQ ID NO: 6 - protein, 315 aa, Bacteroides nordii JCM 12987
MKTIKVKFVDFWENFDPQHNFIANIISKKYRIELSDTPDYLFFSVFGYENIDYHNCTKIFYSGENITPDFNICDYAIGFNFLSFGDRYIRIPFYTAYGVQQLAAPKVIVPEVVLNRKFCSFVVSNAKGAPERERFFQLLSEYKQVDSGGRYKNNVGGPVPDKTAFIKDYKFNIAFENSMCDGYTTEKIMEPMLVNSVPIYWGNKLIDRDFNPASFINVSSYSSLEEAVEHIVRLDQNDDEYLSLLSAPWFNEENYLNWEEQLITFFDNIFEKPLSESRYIPTHGYIQTYQYRLHRMMRDKLFRKRINPLKWFSSK

SEQ ID NO: 7 - DNA, 990 bp, Bacteroides salyersiae JCM 12988
  source 1..990: mol_type = genomic DNA
atgaaaaaagtgaaaattaaatttgtagacttttttgatggctttgataaaggacgcaatgaatttcttgaagtattgaagcaaagatatgagatcgatattagtgatgagcctgattatgtaatatattctggttttggttatgaacatttgaaatataattgtatacgtatattttttacaggagaatgtcaaacacctgacttcaatgagtgtgattatgccataggttttgaccgattaaagtttggtgatcgctatgttcgcattccattatataatatgatgcaatataagttagattataaggaattgttgaatagaaaatctataatatctgatgatatcaaaggacgtggtttttgtagttttgtagtgtcaaattgctttgcaaatgatactcgtgcaatattttatgaattattgaaccaatataaatatatagcttcaggagggagatacaaaaacaatataggtggtgcaataaaggataaaaaaacattcctttcaaagtataagtttaatattgcttttgaaaattgttctcacgatggttatgctacggagaaaatagtggaagcctttgctgcgggggtagtccccatttattatggtgatcctcgtatagcagaagatttcaatcctaaggcatttataaatgctcatgattatcagtcctttgaggagatggttgaacgtataaaggagattgatgcagacgacaggttatatttaacaatgctcaatgaacccataatacaaccgaatgctgatgtaaccgaattggcagattttctttatagtatctttgaccaacctttagcaaaggctaaaagacgctcacaatctcaacctacacaagcaatggaagcgatgaaacttcggcatgagttttttgaaatgaaaatatataaatattataaaaagggcatgaatcaatttacccgcctgaggaagggagtcttcctttcatctaaacgtacaaaataa

SEQ ID NO: 8 - protein, 329 aa, Bacteroides salyersiae JCM 12988
MKKVKIKFVDFFDGFDKGRNEFLEVLKQRYEIDISDEPDYVIYSGFGYEHLKYNCIRIFFTGECQTPDFNECDYAIGFDRLKFGDRYVRIPLYNMMQYKLDYKELLNRKSIISDDIKGRGFCSFVVSNCFANDTRAIFYELLNQYKYIASGGRYKNNIGGAIKDKKTFLSKYKFNIAFENCSHDGYATEKIVEAFAAGVVPIYYGDPRIAEDFNPKAFINAHDYQSFEEMVERIKEIDADDRLYLTMLNEPIIQPNADVTELADFLYSIFDQPLAKAKRRSQSQPTQAMEAMKLRHEFFEMKIYKYYKKGMNQFTRLRKGVFLSSKRTK

SEQ ID NO: 9 - DNA, 1887 bp, Parabacteroides goldsteinii JCM 13446
  source 1..1887: mol_type = genomic DNA
atgagtacttcatgtccttttttatctataatagttccgatatataatgtcgcaacatatctggaagagtgtttgaactctttgatcaacatacggataatttcaaaggagattattttgatcaatgatggctctactgatcggtccggagaaattgcagagaagttcgcttcttctcattcctgtataaagctctttcatcaaccgaatcagggattgtcggcagcacgtaataaaggattgtctgaagtgcaaggggaatatataatgtttatcgacagcgacgattggataatagaaggacagaccgaaaaaatgttctcggaagctatcggttttcaccccgacataataatgggaaattccgtttgttattatcctgacggacaaaccgggaccttatttaatccaatcccatcccatttatgccatacctgcctgacaggaaaagagtgtttttcagaattaatgaaacacggggcttttcctccgatggtttctaattacctatacaaaaaggactggctaaacaagcaaacattgtattttgagaatgttgtccacgaagacgaactctggactccccaagctctttgccttgcaaaaagcatttacatcaccaacattgatttttacggataccggcaacgggaaggttctatcatgaggacattggtcacgtccaaacgcgtacgagacctgatctatatagctaatcgtttgattcgttttgcatcgggataccgtttcaatggcccggaccgggaaatgaaaagcgaactatacgcaaaagcttatatgttatataatttagctttcttatcactggccaaaatcaaaaatggtaatttcactttaccgtcacatgcattgtataccatttttaaaatatatcaccatctctcaccactctcaaaaaagaggatttaccgctattacaaaaatgcccagaataatttgaagagttatttaaaatggaagatatcttactgggcggagaaattatctcctgaaataataaaaaacaaacatattatattgatatataatacgatgtgggatactcctctaaacattcccgttgagcagataccggaaaactataggtttacgactgacagacagtattattctcaggcacaaacagttattttccacttacctactttaatcaatgaattagaaaacgatctggataaacctgaaggacaaatatgggttgcctggacattggaatgcgaagaaaactacccgttcttcaaagatccggaattcatggaactatttgactaccggatttcttatcatcaaacggcagacgtcatacaatcgtatttgcatgacaattttattcctttgatgaaacaaccagtcgacacaaaggagagagccaacaatatctgtatgcttatatccagcccgatcaaccaaagttcgagacaggaatacctgaaagaacttatgcgggaaatacctatagattcctatggaaaactattcaataataagaaaatggatcaggataacggaagggagtccaaaatcaatttatataaacagtacaaatttgttattgcttttgaaaatgcctgtgcaaccgattatgtaacggagaaattctttgatccgttgatcgccggagcggttcccatctatttaggcgcccctaacatcaacgagttcgcacctggagagcattgttttatccatgcaaatgactttaaatcccctaaagagttagccgattatatagaagaatgttacaataatgaacaggaatatcaatcttttttccaatggaaacaaaaagacctccgtcctcaattcatagagaaagcccaattacaaaaaacagctcccttcatccgcttatgtgaacttatttga

SEQ ID NO: 10 - protein, 628 aa, Parabacteroides goldsteinii JCM 13446
MSTSCPFLSIIVPIYNVATYLEECLNSLINIRIISKEIILINDGSTDRSGEIAEKFASSHSCIKLFHQPNQGLSAARNKGLSEVQGEYIMFIDSDDWIIEGQTEKMFSEAIGFHPDIIMGNSVCYYPDGQTGTLFNPIPSHLCHTCLTGKECFSELMKHGAFPPMVSNYLYKKDWLNKQTLYFENVVHEDELWTPQALCLAKSIYITNIDFYGYRQREGSIMRTLVTSKRVRDLIYIANRLIRFASGYRFNGPDREMKSELYAKAYMLYNLAFLSLAKIKNGNFTLPSHALYTIFKIYHHLSPLSKKRIYRYYKNAQNNLKSYLKWKISYWAEKLSPEIIKNKHIILIYNTMWDTPLNIPVEQIPENYRFTTDRQYYSQAQTVIFHLPTLINELENDLDKPEGQIWVAWTLECEENYPFFKDPEFMELFDYRISYHQTADVIQSYLHDNFIPLMKQPVDTKERANNICMLISSPINQSSRQEYLKELMREIPIDSYGKLFNNKKMDQDNGRESKINLYKQYKFVIAFENACATDYVTEKFFDPLIAGAVPIYLGAPNINEFAPGEHCFIHANDFKSPKELADYIEECYNNEQEYQSFFQWKQKDLRPQFIEKAQLQKTAPFIRLCELI

SEQ ID NO: 11 - DNA, 996 bp, Bacteroides fragilis ATCC 25285
  source 1..996: mol_type = genomic DNA
atgtgtgattgcttgtctatcatattgttagtcaaaatgaaaaagatttatttgaaatttgttgatttttgggatggatttgatactatttctaactttattgtggatgctttgtccattcaatacgaagtagtactatctaatgagccagattatttattctattcatgttttggaacgtcacatttagaatatgattgtataaaaatcatgtttataggtgaaaatatagttcctgattttaacgtttgtgattatgccataggttttaattatattgattttggggaccgttacttgaggttgcctttatatgctatatatgatggattttcaaacttgcagaataaaaagattgatgtaaataaagctttagaccgtaaattttgtagtattgttgtttcaaataataaatgggcagatcctattcgtgagactttctttaaattactatctagttataagaaagtagactctggtggaagagcttggaataatataggaggacctgttgataataaattggattttattagccaatataagtttaatattgcttttgaaaatagtagggtactgggatatacaacagaaaaaataatggaacctatgcaggtgaattctattccagtatattggggaaatcctttggttggtaaagattttaatgtggactcctttgtaaatgctcatgattttgattctttagaaagattagttgagtatattatagaattggattcttcaaaggataaatatctggaaatgttggaaaaaccttggcttctcgataagacatatttggattggaaacaattgctgttaaattttattaataatattatgatgaaatcatataaggatgcgaagtatttggttaattatggtcatgctggaaagtatagaaatgaacaacgcttttgggggagatgtgaacgtaaatttaaacttcaaagaattattgaatattattctcaattgtttgatagaaaataa

SEQ ID NO: 12 - protein, 331 aa, Bacteroides fragilis ATCC 25285
MCDCLSIILLVKMKKIYLKFVDFWDGFDTISNFIVDALSIQYEVVLSNEPDYLFYSCFGTSHLEYDCIKIMFIGENIVPDFNVCDYAIGFNYIDFGDRYLRLPLYAIYDGFSNLQNKKIDVNKALDRKFCSIVVSNNKWADPIRETFFKLLSSYKKVDSGGRAWNNIGGPVDNKLDFISQYKFNIAFENSRVLGYTTEKIMEPMQVNSIPVYWGNPLVGKDFNVDSFVNAHDFDSLERLVEYIIELDSSKDKYLEMLEKPWLLDKTYLDWKQLLLNFINNIMMKSYKDAKYLVNYGHAGKYRNEQRFWGRCERKFKLQRIIEYYSQLFDRK

SEQ ID NO: 13 - DNA, 891 bp, Bacteroides fragilis ATCC 25285
  source 1..891: mol_type = genomic DNA
atggatatattgattcttttttataatacgatgtggggatttccactcgagttccgaaaggaagatttacctgggggctgtgtgataacgactgatcgaaacctcattgcaaaggcggatgccgtggttttccatttgcccgatttgccttcggtgatggaggatgaaatcgataagcgggaaggacagctttgggtgggatggagtctggaatgtgaagagaattatagttggacgaaggatcccgagttcagagagagttttgacttatggatggggtatcatcaggaggatgatattgtgtatccttattatggaccggattatgggaagatgctggttacggcacggagggaaaagccttataagaagaaggcatgtatgtttatttcgagtgatatgaaccggagtcaccgacaagagtatcttaaggaattgatgcagtataccgacatcgattcgtatgggaaactataccgtaattgtgaattacctgttgaggatcggggacgggatacacttcttagtgtgatcggggattatcagtttgtgataagttttgagaatgcgatagggaaggattatgtgacagaaaagtttttcaatcctttgttggccggtactgttccggtctatctgggagctcccaatattcgggaatttgctccgggagaaaattgttttctggatatttgtactttcgattctcccgagggagtagccgcttttatgaatcaatgctatgatgacgaggcattgtatgaacgtttttatgcatggaggaaacggcctttattattgtcgtttacaaataagttagagcaagtccggagcaatccgttaatcaggctttgccaaaaaatacacgaactaaaattgggagggatatga

SEQ ID NO: 14 - protein, 296 aa, Bacteroides fragilis ATCC 25285
MDILILFYNTMWGFPLEFRKEDLPGGCVITTDRNLIAKADAVVFHLPDLPSVMEDEIDKREGQLWVGWSLECEENYSWTKDPEFRESFDLWMGYHQEDDIVYPYYGPDYGKMLVTARREKPYKKKACMFISSDMNRSHRQEYLKELMQYTDIDSYGKLYRNCELPVEDRGRDTLLSVIGDYQFVISFENAIGKDYVTEKFFNPLLAGTVPVYLGAPNIREFAPGENCFLDICTFDSPEGVAAFMNQCYDDEALYERFYAWRKRPLLLSFTNKLEQVRSNPLIRLCQKIHELKLGGI

SEQ ID NO: 15 - DNA, 909 bp, Mediterranea sp. An20
  source 1..909: mol_type = genomic DNA
atgcgtaagattctgattctgttctacaataaactgtggggcgttagctgggaaaatgaggcgtgcgcgagcatcccggacggctttgagctgaccgacgatcgtagccgtatggcggaagcggacgcggtggttttccacctgccggacctggcgcgttgcatggatggcgaggaaatcgagaaacgtgatggccagctgtgggtgacctggaacctggaatgcgacgataactacccgtgggttgaggcgccggaaatccgtgacctgttcgatctgcgtattggttatcgtcagcaagacgatgtgtggtacccgtatttcagctttattcgtgcggaggcgtttacccgtctgccgccgcgtcgtccgccgctggacaaggcgtgcctgttcgtgagcagcccgtttaaccgtagccaccgtttcgagtttctgcgtgaactgatgcgtcacaccgaagttgatagcttcggtcgtatgctgcacaacaaagacctgccggcggatgagggccgtaagaccctgatggaaaaaatcgcggactacaagtttgtgattggtgttgagaacgcgctggcgcgtgattatgttaccgaaaagttctttcaaccgctgctggcgggtaccgtgccggtttaccgtggcgcgccgaacgtggaggaatttgcgccgggtcgtcactgcttcgttgacgcgcgtgcgttccgtagcccggcggatctggcgggttttatgaaccgttgctacgagcacccggcgctgtatgacgaactgaccgcgtggcgtacccagccgctgcaaccgggctttgtgcagaaactggagcaagttaaggaacacccgttcgttcgcctgtgccgtgtggttgaggagaaaatccgccgcattgaatacaaaatcacctaa

SEQ ID NO: 16 - protein, 302 aa, Mediterranea sp. An20
MRKILILFYNKLWGVSWENEACASIPDGFELTDDRSRMAEADAVVFHLPDLARCMDGEEIEKRDGQLWVTWNLECDDNYPWVEAPEIRDLFDLRIGYRQQDDVWYPYFSFIRAEAFTRLPPRRPPLDKACLFVSSPFNRSHRFEFLRELMRHTEVDSFGRMLHNKDLPADEGRKTLMEKIADYKFVIGVENALARDYVTEKFFQPLLAGTVPVYRGAPNVEEFAPGRHCFVDARAFRSPADLAGFMNRCYEHPALYDELTAWRTQPLQPGFVQKLEQVKEHPFVRLCRVVEEKIRRIEYKIT

SEQ ID NO: 17 - DNA, 975 bp, Parabacteroides sp. BX2
  source 1..975: mol_type = genomic DNA
atgaaaaaaaagattcgttgttattttactgatttttggaacggttttaattatgaatataccttcaggtttctcttttcggaatatgagtttctgcttgatgaaaaaaatccggactacctgttttatagttgtaatggaaataatcatttggactataatgactgcataaaaattttctggagtgccgagaatgtgatcccggatttgaatttgtgtgactatgcagtgggttcattcgacctgcagagtggagaccggactttacgtgagtttatctacctggcggaaataaataaccggtatattccggaactggatacagaacaactgctgcatcgtaaattctgtaattttgtttataccaataatacatgtgcagatccgatgcgtgaacgtttttttaaggctttgtccaactataaacggatagatgccggtggtggttttttgaataatatgggtaaaagggtcgttaataaacgggctttcctgaaagagtataaatttacgctggcgatagaaaattcgagttttaccggatatacgacagaaaaaatatgtgatccgttcatgagtcaatcgttgccaatttactgggggaacccccatatcagtttggattataatccaaattcgtttgtcaatattatggactattcctctgtggaagaagcggtagaagaggttatccgcctggataatgatgatgacgcctacctggaaaagatgaccgctcctttttggctgtatggaaatagtttcgaagaattttatgcggcaagagtcgaacggatgttggctttcttccggaatatctttgaacagcctctggaaaaagcccgtagacgaacaagatacggaaatgcagaattgtattatttgaccatgaaaaggtattctctttctccggaacggctgttgaaagagaagtatatgaatttattgcgtagagttataaaaaggttacggtga

SEQ ID NO: 18 - protein, 324 aa, Parabacteroides sp. BX2
MKKKIRCYFTDFWNGFNYEYTFRFLFSEYEFLLDEKNPDYLFYSCNGNNHLDYNDCIKIFWSAENVIPDLNLCDYAVGSFDLQSGDRTLREFIYLAEINNRYIPELDTEQLLHRKFCNFVYTNNTCADPMRERFFKALSNYKRIDAGGGFLNNMGKRVVNKRAFLKEYKFTLAIENSSFTGYTTEKICDPFMSQSLPIYWGNPHISLDYNPNSFVNIMDYSSVEEAVEEVIRLDNDDDAYLEKMTAPFWLYGNSFEEFYAARVERMLAFFRNIFEQPLEKARRRTRYGNAELYYLTMKRYSLSPERLLKEKYMNLLRRVIKRLR

SEQ ID NO: 19 - DNA, 996 bp, Parabacteroides sp. HGS0025
  source 1..996: mol_type = genomic DNA
atgaaaaagcaaatacgttattatttcaccgacttctggtctagctttgatttcaaagactgtttttggtatatattttcggaatatgacctgatacttgataaggaacgaccggattacttgttttattcttgttttggaaccgatcatttgttatacgaccgttgtgtaaaaatattctggtcaggagaaaatatgatcccggatctgaatatatgcgactatgcgttcagtttaagtaatatacaatgtgatgatcgtactttcaggcttcgttcggaaggtatgtatagggctaaaggtctgtttgaaacagatctgaaggaggagatgctattacatcgcaaattttgtaattttgtctatggaaataactggtgtgccgatccttatcgattggacttttataagaaattatccggatataaaaagatcgattcagcaggttccttgatgaataatatgaatggtttcaaggtccctgaatgtgagagtaaattatcttttatcagtaaatataaatttactattgccattgaaaattcaagtcaaaatggttattcgacagagaagattgtagaaccatttctggcaaggactttgccgatttattggggtgaccccaatattaatcaggattataatcctgattcttttgttaatctaatgtctttttcttctatcgatgatgctgtcgaagagatcattcgcctggatcaggacgatgaagcttacctgcaaaagatacaagcccctttctggccatacggtaatagctttgaagaattttgtaattgtgagttgaagaaaataatggctttctggcatcatatattcgaccagccgaaagaaaaggcttatcggcgtactatgtatggaaatagcaaaatgtatgtaaataggaagattctggaaaaaagaatgaacatgaagattaaatcgatcggattagataatcgcctaattcgttcggttatgaccagacttttaaaataa

SEQ ID NO: 20 - protein, 331 aa, Parabacteroides sp. HGS0025
MKKQIRYYFTDFWSSFDFKDCFWYIFSEYDLILDKERPDYLFYSCFGTDHLLYDRCVKIFWSGENMIPDLNICDYAFSLSNIQCDDRTFRLRSEGMYRAKGLFETDLKEEMLLHRKFCNFVYGNNWCADPYRLDFYKKLSGYKKIDSAGSLMNNMNGFKVPECESKLSFISKYKFTIAIENSSQNGYSTEKIVEPFLARTLPIYWGDPNINQDYNPDSFVNLMSFSSIDDAVEEIIRLDQDDEAYLQKIQAPFWPYGNSFEEFCNCELKKIMAFWHHIFDQPKEKAYRRTMYGNSKMYVNRKILEKRMNMKIKSIGLDNRLIRSVMTRLLK

SEQ ID NO: 21 - DNA, 993 bp, Parabacteroides bouchesdurhonensis strain Marseille-P3763
  source 1..993: mol_type = genomic DNA
atgaaaagaacaatacgctgcgcatttactgatttggactcttggccaaactttcgtcctccattgcttgaggataattatgaagtgataatagacacggaacatccagattatttattttattcctgttttggcagagagcattataaatataaagattgcgttaaaatattttggtccggagaaaatgtagaacctgattttaatgaatgtgattatgccgcaacctgttcagagtgtgtatatggagatcgggcaatgcgttgttatagcaacgatatttataaatacttaaaaaacggtagagtaaatatattatctaaagaggacttgcttaaccgtaagttttgtaattttatttacggcaataattggtgcgccgatcctttcagggttcgttttttcaatgaattgtctaaatataagaaagtggattcagccggtcctttattaaataatatgggatttaccgttccgcaaggatgggatcctaaaatacagtttcaaagcggatataaattttcattggctatcgaaaattccagtatgccggggtatacaacggaaaaaatacttcatcctttccaggctcattcattgccggtttattgggggaacccccatataagttcggattataatccgaactcgtttgttaatataatgaatttttcgtccgtcgaagaggctgtagaagaaatcatccgcctggataatgacgacgatgcgtaccttgaaaaggtaacggccccgttctggccttatggagacagttttgaagattttcagagccaggagaaaaaacgtcttctcgatttttacgattctatctttaaccaaccgttagaacaggcctatcgcagggctaaatatggatggaataaggtagaacaatcgaaacgacaaagattggaattgcctcaacctttgctttccatcgtgaaaagtagagtgaaaagaaaattgaaaggggggtggacaaatttgggatag

SEQ ID NO: 22 - protein, 330 aa, Parabacteroides bouchesdurhonensis strain Marseille-P3763
MKRTIRCAFTDLDSWPNFRPPLLEDNYEVIIDTEHPDYLFYSCFGREHYKYKDCVKIFWSGENVEPDFNECDYAATCSECVYGDRAMRCYSNDIYKYLKNGRVNILSKEDLLNRKFCNFIYGNNWCADPFRVRFFNELSKYKKVDSAGPLLNNMGFTVPQGWDPKIQFQSGYKFSLAIENSSMPGYTTEKILHPFQAHSLPVYWGNPHISSDYNPNSFVNIMNFSSVEEAVEEIIRLDNDDDAYLEKVTAPFWPYGDSFEDFQSQEKKRLLDFYDSIFNQPLEQAYRRAKYGWNKVEQSKRQRLELPQPLLSIVKSRVKRKLKGGWTNLG

SEQ ID NO: 23 - DNA, 966 bp, Gramella sp. BOM4
  source 1..966: mol_type = genomic DNA
atgaaaaatataaaaatctggtttaccgatttctaccaaggttttcaaccttcagataatccatttataaatatattaaaggaccgattttctgtagaattggacagcgattctcctgatttcttattctactcctgttacggatatgattttctccactataattgcccccggattttttacacaggggaaaaccttaggcctgattttaatctatgtgattacgcaataggctttgaccattttgaattcgaagacaggtatctccgatttcctaattatgccttattcgaaggacagtttgaaaagttaacagagataaaaaatgatggaatcgaagataaagattatttctgcaatttcatttattcaaataatcaggcaaatcctattcgcgatcaatttttccattctttaaatgaatataaaaagatcagttctcccggaaaacatctgaacaatgtaaacattgagattggcgggagatatgcctcggactggatgttcagcaaaatagattttcaatcgaaatgcaaattcaccattgcttttgaaaacagttcttcaccggggtatactacggaaaagatcatgcatgcatttttggcaggcactattcccatttactggggaaaccctaaagtaaaccttgattttaatcccgaagcttttatcaattatcacgattttaataatctgcaggagcttaaaagtgaagtgattagagtagatcaggataaagagttatatgaggagattatgaaaaagcctgttttcaggaataatatgatgcctgaaaatcttaaaaaggaacgattaattgaattccttcaatcaattctaaatcagaatctcgaatctgcctttagaagacctcgatacggtactactattaaatatgagtctaggttaaaagaaatgatccgaaaaaaaaattcattcaaatggaagaagcttttcaggtag

SEQ ID NO: 24 - protein, 321 aa, Gramella sp. BOM4
MKNIKIWFTDFYQGFQPSDNPFINILKDRFSVELDSDSPDFLFYSCYGYDFLHYNCPRIFYTGENLRPDFNLCDYAIGFDHFEFEDRYLRFPNYALFEGQFEKLTEIKNDGIEDKDYFCNFIYSNNQANPIRDQFFHSLNEYKKISSPGKHLNNVNIEIGGRYASDWMFSKIDFQSKCKFTIAFENSSSPGYTTEKIMHAFLAGTIPIYWGNPKVNLDFNPEAFINYHDFNNLQELKSEVIRVDQDKELYEEIMKKPVFRNNMMPENLKKERLIEFLQSILNQNLESAFRRPRYGTTIKYESRLKEMIRKKNSFKWKKLFR

SEQ ID NO: 25 - DNA, 1002 bp, Lachnospiraceae bacterium NLAE-zl-G231
  source 1..1002: mol_type = genomic DNA
atgaaagaaataaaagttaaatttgttgactattgggatgatcatcatttggaaaaagatataatttataagatattaaaaaaacattatcaggtaaaaatagttgaggatccggattatttattctattcagttttttctgatgataatctaaaatatgattgtattaaaatcttttatactgcggaaaatatttgtcctgattttaacctatgtgattatgcaattggatttgaagaattacaatttagtgatagatatattagaatacctaatttcgttaaatatttatctgatattgaactgatgaaaaataaaaataaagatattattaatgatgaagattttttaaatagaaaattttgtagttttatatattcaaatggaaatgctgatattaaaagagaaaagttattttatgaaatttccaaatataaaaaaattaactcggctggtcgttacttaaataatgtaggtaaagttattgaagataaaattgattatgaaaaaaattttaaattttcaatagcttgtgaaaattgttcacatatggggtatagtactgaaaaaatagttcaatcatttgcggctaaaacagttcctatatactggggagatcctgatattgataaggtttttaatccgaaatcttttattaatttgatgaagtttagtgattttaacgaagctatacaatatattaaaaatgttgatgcaaacggaagtttatatttaaatatgttaagagagccggctttgttagacccaacatactgtgataagaagtatatggagttggaaagctttttggtgaatattatagagcaacctaaagatgaggcctatcgtcgttgtaacattgccagaatgggtgaatatcaacgaaaaatggaagagtggcgaaatatatatttaatgagaaaatataaggaagaacataatattgtaaataaaattgtaaatttaagcaaaacatttttggataaattcttggttaattaa

SEQ ID NO: 26 - protein, 333 aa, Lachnospiraceae bacterium NLAE-zl-G231
MKEIKVKFVDYWDDHHLEKDIIYKILKKHYQVKIVEDPDYLFYSVFSDDNLKYDCIKIFYTAENICPDFNLCDYAIGFEELQFSDRYIRIPNFVKYLSDIELMKNKNKDIINDEDFLNRKFCSFIYSNGNADIKREKLFYEISKYKKINSAGRYLNNVGKVIEDKIDYEKNFKFSIACENCSHMGYSTEKIVQSFAAKTVPIYWGDPDIDKVFNPKSFINLMKFSDFNEAIQYIKNVDANGSLYLNMLREPALLDPTYCDKKYMELESFLVNIIEQPKDEAYRRCNIARMGEYQRKMEEWRNIYLMRKYKEEHNIVNKIVNLSKTFLDKFLVN

SEQ ID NO: 27 - DNA, 1233 bp, E. coli W3110
  source 1..1233: mol_type = genomic DNA
atgcaaaataaattagcttccggtgccaggcttggacgtcaggcgttacttttccctctctgtctggtgctttacgaattttcaacctatatcggcaacgatatgattcaacccggtatgttggccgtggtggaacaatatcaggcgggcattgattgggttcctacttcgatgaccgcgtatctggcgggcgggatgtttttacaatggctgctggggccgctgtcggatcgtattggtcgccgtccggtgatgctggcgggagtggtgtggtttatcgtcacctgtctggcaatattgctggcgcaaaacattgaacaattcaccctgttgcgcttcttgcagggcataagcctctgtttcattggcgctgtgggatacgccgcaattcaggaatccttcgaagaggcggtttgtatcaagatcaccgcgctgatggcgaacgtggcgctgattgctccgctacttggtccgctggtgggcgcggcgtggatccatgtgctgccctgggaggggatgtttgttttgtttgccgcattggcagcgatctcctttttcggtctgcaacgagccatgcctgaaaccgccacgcgtataggcgagaaactgtcactgaaagaactcggtcgtgactataagctggtgctgaagaacggccgctttgtggcgggggcgctggcgctgggattcgttagtctgccgttgctggcgtggatcgcccagtcgccgattatcatcattaccggcgagcagttgagcagctatgaatatggcttgctgcaagtgcctattttcggggcgttaattgcgggtaacttgctgttagcgcgtctgacctcgcgccgcaccgtacgttcgctgattattatgggcggctggccgattatgattggtctattggtcgctgctgcggcaacggttatctcatcgcacgcgtatttatggatgactgccgggttaagtatttatgctttcggtattggtctggcgaatgcgggactggtgcgattaaccctgtttgccagcgatatgagtaaaggtacggtttctgccgcgatgggaatgctgcaaatgctgatctttaccgttggtattgaaatcagcaaacatgcctggctgaacgggggcaacggactgtttaatctcttcaaccttgtcaacggaattttgtggctgtcgctgatggttatctttttaaaagataaacagatgggaaattctcacgaagggtaa

SEQ ID NO: 28 - protein, 410 aa, E. coli W3110
MQNKLASGARLGRQALLFPLCLVLYEFSTYIGNDMIQPGMLAVVEQYQAGIDWVPTSMTAYLAGGMFLQWLLGPLSDRIGRRPVMLAGVVWFIVTCLAILLAQNIEQFTLLRFLQGISLCFIGAVGYAAIQESFEEAVCIKITALMANVALIAPLLGPLVGAAWIHVLPWEGMFVLFAALAAISFFGLQRAMPETATRIGEKLSLKELGRDYKLVLKNGRFVAGALALGFVSLPLLAWIAQSPIIIITGEQLSSYEYGLLQVPIFGALIAGNLLLARLTSRRTVRSLIIMGGWPIMIGLLVAAAATVISSHAYLWMTAGLSIYAFGIGLANAGLVRLTLFASDMSKGTVSAAMGMLQMLIFTVGIEISKHAWLNGGNGLFNLFNLVNGILWLSLMVIFLKDKQMGNSHEG

SEQ ID NO: 29 - DNA, 822 bp, Helicobacter pylori NCTC 11637
  source 1..822: mol_type = genomic DNA
atgcgtgtttttatcatttctttaaatcaaaaagtgtgcgatacatttggtttggtttttagagacaccacgactttactcaataatattaatgccacccaccaccaagcgcaaatttttgatgcgatttattctaaaacttttgaaggcgggttgcaccccttagtgaaaaagcatttacacccttatttcatcacgcaaaacatcaaagacatggggattacaaccaatctcatcagtgaggtttctaagttttattacgctttaaaataccatgcgaagtttatgagcttgggggagcttgggtgctatgcgagccattattccttgtgggaaaaatgcatagaactcaatgaagcgatctgtattttagaagacgatataaccttaaaagaggattttaaagagggattggattttttagaaaaacacatccaagagttaggctatgttcgcttgatgcatttattatatgaccccaatgttaaaagtgagccattgaaccataaaaaccacgagatacaagagcgtgtggggatcattaaagcttatagtcatggggtggggacgcaaggctatgtgatcacgcccaagattgccaaagtttttaaaaaacacagccgaaaatgggttgttcctgtggatacgataatggacgctacttttatccatggcgtgaaaaatctggtgttacaaccttttgtgatcgctgatgatgagcagatctctacgatagcacgaaaagaagaaccttatagccctaaaatcgccttaatgagagaactccattttaaatatttgaaatattggcagtttgtatag

SEQ ID NO: 30 - protein, 273 aa, Helicobacter pylori NCTC 11637
MRVFIISLNQKVCDTFGLVFRDTTTLLNNINATHHQAQIFDAIYSKTFEGGLHPLVKKHLHPYFITQNIKDMGITTNLISEVSKFYYALKYHAKFMSLGELGCYASHYSLWEKCIELNEAICILEDDITLKEDFKEGLDFLEKHIQELGYVRLMHLLYDPNVKSEPLNHKNHEIQERVGIIKAYSHGVGTQGYVITPKIAKVFKKHSRKWVVPVDTIMDATFIHGVKNLVLQPFVIADDEQISTIARKEEPYSPKIALMRELHFKYLKYWQFV

SEQ ID NO: 31 - DNA, 1041 bp, Neisseria polysaccharea ATCC 43768
  source 1..1041: mol_type = genomic DNA
atgcagccgctggtgagcgttctgatttgcgcgtacaacgtggagaagtattttgcgcaggcgctggatgcggtggttggtcaaacctggcgtaacctggacatcctgattgttgacgatggcagcaccgatggtaccctggcgatcgcgaaggactttcaaaaacgtgatagccgtatcaagattctggcgcaggcgcaaaacagcggcctgatcccgagcctgaacattggtctggatgagctggcgaaaagcggtggcggtgaatacattgcgcgtaccgatgcggatgatattgcggcgccggattggatcgagaagattgtgggcgagatggaaaaagaccgtagcatcattgcgatgggtgcgtggctggaagttctgagcgaggaaaaggatggcaaccgtctggcgcgtcaccacgagcacggtaaaatttggaagaaaccgacccgtcacgaagacatcgcggcgttctttccgttcggcaacccgatccacaacaacaccatgattatgcgtcgtagcgtgatcgacggcggtctgcgttacaacaccgagcgtgactgggcggaagattaccagttttggtatgatgttagcaagctgggtcgtctggcgtactatccggaggcgctggtgaagtatcgtctgcacgcgaaccaagttagcagcaaacacagcattcgtcaacacgaaatcgcgcagggcattcaaaagaccgcgcgtaacgacttcctgcagagcatgggtttcaaaacccgttttgatagcctggagtaccgtcaaaccaaggcggcggcgtatgagctgctggaaaaagacctgccggaggaagatttcgaacgtgcgcgtcgtttcctgtaccagtgctttaaacgtaccgacaccccgccggcgggtgcgtggctggactttgcggcggatggtcgtatgcgtcgtctgttcaccctgcgtcaatattttagcatcctgcaccgtctgattaagaaccgtcgtcaggcgcgtagcgatagcgcgggtaaagagcaagaaatctaa

SEQ ID NO: 32 - protein, 346 aa, Neisseria polysaccharea ATCC 43768
MQPLVSVLICAYNVEKYFAQALDAVVGQTWRNLDILIVDDGSTDGTLAIAKDFQKRDSRIKILAQAQNSGLIPSLNIGLDELAKSGGGEYIARTDADDIAAPDWIEKIVGEMEKDRSIIAMGAWLEVLSEEKDGNRLARHHEHGKIWKKPTRHEDIAAFFPFGNPIHNNTMIMRRSVIDGGLRYNTERDWAEDYQFWYDVSKLGRLAYYPEALVKYRLHANQVSSKHSIRQHEIAQGIQKTARNDFLQSMGFKTRFDSLEYRQTKAAAYELLEKDLPEEDFERARRFLYQCFKRTDTPPAGAWLDFAADGRMRRLFTLRQYFSILHRLIKNRRQARSDSAGKEQEI

SEQ ID NO: 33 - DNA, 20 bp, synthetic construct
  misc_feature 1..20: note = Description of the artificial sequence: base sequence of primer for amplification of catsacB fragment
  source 1..20: mol_type = other DNA
accaggcgtttaagggcacc

SEQ ID NO: 34 - DNA, 21 bp, synthetic construct
  misc_feature 1..21: note = Description of the artificial sequence: base sequence of primer for amplification of catsacB fragment
  source 1..21: mol_type = other DNA
tacggttagccatttgcctgc

SEQ ID NO: 35 - DNA, 42 bp, synthetic construct
  misc_feature 1..42: note = Description of the artificial sequence: base sequence of primer for amplification of lacZ upstream 1
  source 1..42: mol_type = other DNA
ggtgcccttaaacgcctggtagctgtttcctgtgtgaaattg

SEQ ID NO: 36 - DNA, 18 bp, synthetic construct
  misc_feature 1..18: note = Description of the artificial sequence: base sequence of primer for amplification of lacZ upstream 1
  source 1..18: mol_type = other DNA
ccagtctggccctgcacg

SEQ ID NO: 37 - DNA, 43 bp, synthetic construct
  misc_feature 1..43: note = Description of the artificial sequence: base sequence of primer for amplification of lacY downstream 1
  source 1..43: mol_type = other DNA
gcaggcaaatggctaaccgtacgaccaacatatcataacggag

SEQ ID NO: 38 - DNA, 20 bp, synthetic construct
  misc_feature 1..20: note = Description of the artificial sequence: base sequence of primer for amplification of lacY downstream 1
  source 1..20: mol_type = other DNA
gtttccgctctgtttgctgc

SEQ ID NO: 39 - DNA, 42 bp, synthetic construct
  misc_feature 1..42: note = Description of the artificial sequence: base sequence of primer for amplification of lacZ upstream 2
  source 1..42: mol_type = other DNA
ccgttatgatatgttggtcgagctgtttcctgtgtgaaattg

SEQ ID NO: 40 - DNA, 22 bp, synthetic construct
  misc_feature 1..22: note = Description of the artificial sequence: base sequence of primer for amplification of lacY downstream 2
  source 1..22: mol_type = other DNA
cgaccaacatatcataacggag

SEQ ID NO: 41 - DNA, 41 bp, synthetic construct
  misc_feature 1..41: note = Description of the artificial sequence: base sequence of primer for amplification of wcaJ upstream 1
  source 1..41: mol_type = other DNA
ggtgcccttaaacgcctggtcgttgttcctgttattagccc

SEQ ID NO: 42 - DNA, 20 bp, synthetic construct
  misc_feature 1..20: note = Description of the artificial sequence: base sequence of primer for amplification of wcaJ upstream 1
  source 1..20: mol_type = other DNA
acgcggtcgctatcagcaaa

SEQ ID NO: 43 - DNA, 44 bp, synthetic construct
  misc_feature 1..44: note = Description of the artificial sequence: base sequence of primer for amplification of wcaM downstream 1
  source 1..44: mol_type = other DNA
gcaggcaaatggctaaccgtaatttgcgaccattcctggaaaaa

SEQ ID NO: 44 - DNA, 23 bp, synthetic construct
  misc_feature 1..23: note = Description of the artificial sequence: base sequence of primer for amplification of wcaM downstream 1
  source 1..23: mol_type = other DNA
acttcacaaacgcctgcatatag

SEQ ID NO: 45 - DNA, 41 bp, synthetic construct
  misc_feature 1..41: note = Description of the artificial sequence: base sequence of primer for amplification of wcaJ upstream 2
  source 1..41: mol_type = other DNA
ttccaggaatggtcgcaaatcgttgttcctgttattagccc

SEQ ID NO: 46 - DNA, 23 bp, synthetic construct
  misc_feature 1..23: note = Description of the artificial sequence: base sequence of primer for amplification of wcaM downstream 2
  source 1..23: mol_type = other DNA
atttgcgaccattcctggaaaaa

SEQ ID NO: 47 - DNA, 39 bp, synthetic construct
  misc_feature 1..39: note = Description of the artificial sequence: base sequence of primer for amplification of mdfA fragment
  source 1..39: mol_type = other DNA
acacaggaaacagctatgcaaaataaattagcttccggt

SEQ ID NO: 48 - DNA, 36 bp, synthetic construct
  misc_feature 1..36: note = Description of the artificial sequence: base sequence of primer for amplification of mdfA fragment
  source 1..36: mol_type = other DNA
gggtaacgccagggtttacccttcgtgagaatttcc

SEQ ID NO: 49 - DNA, 20 bp, synthetic construct
  misc_feature 1..20: note = Description of the artificial sequence: base sequence of primer for amplification of pMW118 fragment
  source 1..20: mol_type = other DNA
agctgtttcctgtgtgaaat

SEQ ID NO: 50 - DNA, 18 bp, synthetic construct
  misc_feature 1..18: note = Description of the artificial sequence: base sequence of primer for amplification of pMW118 fragment
  source 1..18: mol_type = other DNA
accctggcgttacccaac

SEQ ID NO: 51 - DNA, 24 bp, synthetic construct
  misc_feature 1..24: note = Description of the artificial sequence: base sequence of primer for amplification of pUAKQE fragment
  source 1..24: mol_type = other DNA
ggttaatttctcctctttaatatc

SEQ ID NO: 52 - DNA, 22 bp, synthetic construct
  misc_feature 1..22: note = Description of the artificial sequence: base sequence of primer for amplification of pUAKQE fragment
  source 1..22: mol_type = other DNA
catcaccatcaccatcactaag

SEQ ID NO: 53 - DNA, 36 bp, synthetic construct
  misc_feature 1..36: note = Description of the artificial sequence: base sequence of primer for amplification of rcsA fragment
  source 1..36: mol_type = other DNA
gaggagaaattaaccgcattgagtgagggtatgcca

SEQ ID NO: 54 - DNA, 44 bp, synthetic construct
  misc_feature 1..44: note = Description of the artificial sequence: base sequence of primer for amplification of rcsA fragment
  source 1..44: mol_type = other DNA
aatggatttccttacgcgaattagcgcatgttgacaaaaatacc

SEQ ID NO: 55 - DNA, 23 bp, synthetic construct
  misc_feature 1..23: note = Description of the artificial sequence: base sequence of primer for amplification of lacY fragment
  source 1..23: mol_type = other DNA
ttcgcgtaaggaaatccattatg

SEQ ID NO: 56 - DNA, 38 bp, synthetic construct
  misc_feature 1..38: note = Description of the artificial sequence: base sequence of primer for amplification of lacY fragment
  source 1..38: mol_type = other DNA
atggtgatggtgatgttaagcgacttcattcacctgac

SEQ ID NO: 57 - DNA, 21 bp, synthetic construct
  misc_feature 1..21: note = Description of the artificial sequence: base sequence of primer for amplification of pUAKQE-rcsA-lacY fragment
  source 1..21: mol_type = other DNA
gcattgagtgagggtatgcca

SEQ ID NO: 58 - DNA, 37 bp, synthetic construct
  misc_feature 1..37: note = Description of the artificial sequence: base sequence of primer for amplification of HpFutA fragment
  source 1..37: mol_type = other DNA
gaggagaaattaaccatgttccaacccctattagacg

SEQ ID NO: 59 - DNA, 40 bp, synthetic construct
  misc_feature 1..40: note = Description of the artificial sequence: base sequence of primer for amplification of HpFutA fragment
  source 1..40: mol_type = other DNA
accctcactcaatgcttacaaacccaattttttaaccaac

SEQ ID NO: 60 - DNA, 42 bp, synthetic construct
  misc_feature 1..42: note = Description of the artificial sequence: base sequence of primer for amplification of BnFucT fragment
  source 1..42: mol_type = other DNA
gaggagaaattaaccatgaaaactataaaagtaaaattcgtt

SEQ ID NO: 61 - DNA, 39 bp, synthetic construct
  misc_feature 1..39: note = Description of the artificial sequence: base sequence of primer for amplification of BnFucT fragment
  source 1..39: mol_type = other DNA
accctcactcaatgctcacttcgaagaaaaccatttcag

SEQ ID NO: 62 - DNA, 42 bp, synthetic construct
  misc_feature 1..42: note = Description of the artificial sequence: base sequence of primer for amplification of BsFucT fragment
  source 1..42: mol_type = other DNA
gaggagaaattaaccatgaaaaaagtgaaaattaaatttgta

SEQ ID NO: 63 - DNA, 40 bp, synthetic construct
  misc_feature 1..40: note = Description of the artificial sequence: base sequence of primer for amplification of BsFucT fragment
  source 1..40: mol_type = other DNA
accctcactcaatgcttattttgtacgtttagatgaaagg

SEQ ID NO: 64 - DNA, 40 bp, synthetic construct
  misc_feature 1..40: note = Description of the artificial sequence: base sequence of primer for amplification of PgsFucT1 fragment
  source 1..40: mol_type = other DNA
gaggagaaattaaccatgaaaaagaaaatatactgcaact

SEQ ID NO: 65 - DNA, 41 bp, synthetic construct
  misc_feature 1..41: note = Description of the artificial sequence: base sequence of primer for amplification of PgsFucT1 fragment
  source 1..41: mol_type = other DNA
accctcactcaatgcttatttctttttcaatagttttttgg

SEQ ID NO: 66 - DNA, 39 bp, synthetic construct
  misc_feature 1..39: note = Description of the artificial sequence: base sequence of primer for amplification of PgsFucT2 fragment
  source 1..39: mol_type = other DNA
gaggagaaattaaccatgagtacttcatgtcctttttta

SEQ ID NO: 67 - DNA, 38 bp, synthetic construct
  misc_feature 1..38: note = Description of the artificial sequence: base sequence of primer for amplification of PgsFucT2 fragment
  source 1..38: mol_type = other DNA
accctcactcaatgctcaaataagttcacataagcgga

SEQ ID NO: 68 - DNA, 40 bp, synthetic construct
  misc_feature 1..40: note = Description of the artificial sequence: base sequence of primer for amplification of BfFucT1 fragment
  source 1..40: mol_type = other DNA
gaggagaaattaaccatgtgtgattgcttgtctatcatat

SEQ ID NO: 69 - DNA, 40 bp, synthetic construct
  misc_feature 1..40: note = Description of the artificial sequence: base sequence of primer for amplification of BfFucT1 fragment
  source 1..40: mol_type = other DNA
accctcactcaatgcttattttctatcaaacaattgagaa

SEQ ID NO: 70 - DNA, 43 bp, synthetic construct
  misc_feature 1..43: note = Description of the artificial sequence: base sequence of primer for amplification of BfFucT2 fragment
  source 1..43: mol_type = other DNA
gaggagaaattaaccatggatatattgattcttttttataata

SEQ ID NO: 71 - DNA, 39 bp, synthetic construct
  misc_feature 1..39: note = Description of the artificial sequence: base sequence of primer for amplification of BfFucT2 fragment
  source 1..39: mol_type = other DNA
accctcactcaatgctcatatccctcccaattttagttc

SEQ ID NO: 72 - DNA, 39 bp, synthetic construct
  misc_feature 1..39: note = Description of the artificial sequence: base sequence of primer for amplification of MFucT fragment
  source 1..39: mol_type = other DNA
gaggagaaattaaccatgcgtaagattctgattctgttc

SEQ ID NO: 73 - DNA, 39 bp, synthetic construct
  misc_feature 1..39: note = Description of the artificial sequence: base sequence of primer for amplification of MFucT fragment
  source 1..39: mol_type = other DNA
accctcactcaatgcttaggtgattttgtattcaatgcg

SEQ ID NO: 74 - DNA, 43 bp, synthetic construct
  misc_feature 1..43: note = Description of the artificial sequence: base sequence of primer for amplification of FucT-A fragment
  source 1..43: mol_type = other DNA
gaggagaaattaaccatgaaaaaaaagattcgttgttatttta

SEQ ID NO: 75 - DNA, 40 bp, synthetic construct
  misc_feature 1..40: note = Description of the artificial sequence: base sequence of primer for amplification of FucT-A fragment
  source 1..40: mol_type = other DNA
accctcactcaatgctcaccgtaacctttttataactcta

SEQ ID NO: 76 - DNA, 42 bp, synthetic construct
  misc_feature 1..42: note = Description of the artificial sequence: base sequence of primer for amplification of FucT-B fragment
  source 1..42: mol_type = other DNA
gaggagaaattaaccatgaaaaagcaaatacgttattatttc

SEQ ID NO: 77 - DNA, 40 bp, synthetic construct
  misc_feature 1..40: note = Description of the artificial sequence: base sequence of primer for amplification of FucT-B fragment
  source 1..40: mol_type = other DNA
accctcactcaatgcttattttaaaagtctggtcataacc

SEQ ID NO: 78 - DNA, 38 bp, synthetic construct
  misc_feature 1..38: note = Description of the artificial sequence: base sequence of primer for amplification of FucT-C fragment
  source 1..38: mol_type = other DNA
gaggagaaattaaccatgaaaagaacaatacgctgcgc

SEQ ID NO: 79 - DNA, 37 bp, synthetic construct
  misc_feature 1..37: note = Description of the artificial sequence: base sequence of primer for amplification of FucT-C fragment
  source 1..37: mol_type = other DNA
accctcactcaatgcctatcccaaatttgtccacccc

SEQ ID NO: 80 - DNA, 42 bp, synthetic construct
  misc_feature 1..42: note = Description of the artificial sequence: base sequence of primer for amplification of FucT-D fragment
  source 1..42: mol_type = other DNA
gaggagaaattaaccatgaaaaatataaaaatctggtttacc

SEQ ID NO: 81 - DNA, 38 bp, synthetic construct
  misc_feature 1..38: note = Description of the artificial sequence: base sequence of primer for amplification of FucT-D fragment
  source 1..38: mol_type = other DNA
accctcactcaatgcctacctgaaaagcttcttccatt

SEQ ID NO: 82 - DNA, 43 bp, synthetic construct
  misc_feature 1..43: note = Description of the artificial sequence: base sequence of primer for amplification of FucT-E fragment
  source 1..43: mol_type = other DNA
gaggagaaattaaccatgaaagaaataaaagttaaatttgttg

SEQ ID NO: 83 - DNA, 44 bp, synthetic construct
  misc_feature 1..44: note = Description of the artificial sequence: base sequence of primer for amplification of FucT-E fragment
  source 1..44: mol_type = other DNA
accctcactcaatgcttaattaaccaagaatttatccaaaaatg

SEQ ID NO: 84 - DNA, 45 bp, synthetic construct
  misc_feature 1..45: note = Description of the artificial sequence: base sequence of primer for amplification of PgsFucT1 N17D upstream
  source 1..45: mol_type = other DNA
cagaaataagttttataatcaaaaccaagccaaaaatcaacaaag

SEQ ID NO: 85 - DNA, 29 bp, synthetic construct
  misc_feature 1..29: note = Description of the artificial sequence: base sequence of primer for amplification of PgsFucT1 N17D downstream
  source 1..29: mol_type = other DNA
gattataaaacttatttctggtatttgtc

SEQ ID NO: 86 - DNA, 44 bp, synthetic construct
  misc_feature 1..44: note = Description of the artificial sequence: base sequence of primer for amplification of PgsFucT1 S93L upstream
  source 1..44: mol_type = other DNA
tttctgtacagaaatcccagatatttccgaaaagttctgtcatc

SEQ ID NO: 87 - DNA, 26 bp, synthetic construct
  misc_feature 1..26: note = Description of the artificial sequence: base sequence of primer for amplification of PgsFucT1 S93L downstream
  source 1..26: mol_type = other DNA
ctgggatttctgtacagaaaggattt

SEQ ID NO: 88 - DNA, 44 bp, synthetic construct
  misc_feature 1..44: note = Description of the artificial sequence: base sequence of primer for amplification of BfFucT D28N upstream
  source 1..44: mol_type = other DNA
ataaagttagaaatagtgttaaatccatcccaaaaatcaacaaa

SEQ ID NO: 89 - DNA, 28 bp, synthetic construct
  misc_feature 1..28: note = Description of the artificial sequence: base sequence of primer for amplification of BfFucT D28N downstream
  source 1..28: mol_type = other DNA
aacactatttctaactttattgtggatg

SEQ ID NO: 90 - DNA, 41 bp, synthetic construct
  misc_feature 1..41: note = Description of the artificial sequence: base sequence of primer for amplification of BfFucT L104S upstream
  source 1..41: mol_type = other DNA
ccatcatatatagcatagctaggcaacctcaagtaacggtc

SEQ ID NO: 91 - DNA, 28 bp, synthetic construct
  misc_feature 1..28: note = Description of the artificial sequence: base sequence of primer for amplification of BfFucT L104S downstream
  source 1..28: mol_type = other DNA
agctatgctatatatgatggattttcaa

SEQ ID NO: 92 - DNA, 22 bp, synthetic construct
  misc_feature 1..22: note = Description of the artificial sequence: base sequence of primer for amplification of pSTV29 fragment
  source 1..22: mol_type = other DNA
agctgtttcctgtgtgaaattg

SEQ ID NO: 93 - DNA, 20 bp, synthetic construct
  misc_feature 1..20: note = Description of the artificial sequence: base sequence of primer for amplification of pSTV29 fragment
  source 1..20: mol_type = other DNA
gaattcactggccgtcgttt

SEQ ID NO: 94 - DNA, 41 bp, synthetic construct
  misc_feature 1..41: note = Description of the artificial sequence: base sequence of primer for amplification of HpgalT fragment
  source 1..41: mol_type = other DNA
acacaggaaacagctatgcgtgtttttatcatttctttaaa

SEQ ID NO: 95 - DNA, 61 bp, synthetic construct
  misc_feature 1..61: note = Description of the artificial sequence: base sequence of primer for amplification of HpgalT fragment
  source 1..61: mol_type = other DNA
caccagcggctgcatggttaatttctcctctttaatctatacaaactgccaatatttcaaa

SEQ ID NO: 96 - DNA, 19 bp, synthetic construct
  misc_feature 1..19: note = Description of the artificial sequence: base sequence of primer for amplification of NplgtA fragment
  source 1..19: mol_type = other DNA
atgcagccgctggtgagcg

SEQ ID NO: 97 - DNA, 38 bp, synthetic construct
  misc_feature 1..38: note = Description of the artificial sequence: base sequence of primer for amplification of NplgtA fragment
  source 1..38: mol_type = other DNA
acggccagtgaattcttagatttcttgctctttacccg